European Patent Specification EP 3 597 756 B1, published December 13, 2023. Title: XMP-producing microorganism and method of producing XMP using the same. Applicant: CJ CheilJedang Corporation. The sequence listing filed with the application follows.

SEQUENCE LISTING (21 sequences)

SEQ ID NO: 1 - DNA, 1242 bp, Corynebacterium sp.
gtgcacacaaccgaagaggtcaaactctttacgccgacgtttatcatggggtgggtcgccaacttcctgcagttcttggtgttctacttcctcatcaccacgatggcgctctacgcaaccaaggaattcagcgcatcggaaaccgaagcaggctttgccgccagtgcgattgttatcggtgcggtcttttcccgtttggtttccggatacattattgaccgcttcggtcgccgcaaaattgtggtggtctccgtcatcgcgaccactattgcgtgcgcgctatatatcccgatcgattctttggggctgctctacgctgaccgcttcttccacggtgtagcttatgcctttgcgtgcaccgcgattatggcgatggtccaggaactcattccttctgcacgccgctccgaaggcactggctacctggctttgggtaccaccgtttcggctgctatcggaccagcgctagcgctatttttgctgggttctttcaactacgaagtcctcttcgttgtcgtcctcggcatttcgattgtctctttgatcgcttcgctagtcatctatttccgcacctccgacccagagccagagctggatgaaaacggcaatgctgctgagcccattaagttcagcttcaagtccatcattaaccctaaagtcttgccgattggcctcttcatgctgctggtagcctttgcctactccggcgtgatcgcacatatcaacgcttttgctgaaaaccgcgacgttgttactggcgcaggcctattctttatcgcttacgccatctccatgttcgtgatgcgctcctaccttggtaaattgcaagaccgccggggcgataacagcgttatctactttggtctcgtattctttgttatctcatttatcgtgctctcgctttctaccgccaactggcatgtcgttgtcgctggcgtgctagcaggtctgggctacggcaccttgatgccagctgctcaagcagtatctgttggtgttgtcgacaagagcgagttcggctcagcattttccaccttgttccttttcgttgacctcggcttcggcttcggcccagtcatccttggtgcagtggtttccgcgattggctacggttcgatgtatgcagtgctcgtcggcgtcggcgttattgctggcatctactacctgttcacccacgcacgcaccgagcgcgcaaagcacggcgtagtcaagcatgtagaaaccatggttctggctcaataa

SEQ ID NO: 2 - protein, 413 aa, Corynebacterium sp.
VHTTEEVKLFTPTFIMGWVANFLQFLVFYFLITTMALYATKEFSASETEAGFAASAIVIGAVFSRLVSGYIIDRFGRRKIVVVSVIATTIACALYIPIDSLGLLYADRFFHGVAYAFACTAIMAMVQELIPSARRSEGTGYLALGTTVSAAIGPALALFLLGSFNYEVLFVVVLGISIVSLIASLVIYFRTSDPEPELDENGNAAEPIKFSFKSIINPKVLPIGLFMLLVAFAYSGVIAHINAFAENRDVVTGAGLFFIAYAISMFVMRSYLGKLQDRRGDNSVIYFGLVFFVISFIVLSLSTANWHVVVAGVLAGLGYGTLMPAAQAVSVGVVDKSEFGSAFSTLFLFVDLGFGFGPVILGAVVSAIGYGSMYAVLVGVGVIAGIYYLFTHARTERAKHGVVKHVETMVLAQ

SEQ ID NO: 3 - DNA, 21 bp, Artificial Sequence
  xmpE del F
gtcaaactctttacgccgacg

SEQ ID NO: 4 - DNA, 22 bp, Artificial Sequence
  xmpE del R
cgacaacaccaacagatactgc

SEQ ID NO: 5 - DNA, 31 bp, Artificial Sequence
  xmpE 2copy F (xbaI)
atgctctagactagatcttctcgacgggcag

SEQ ID NO: 6 - DNA, 32 bp, Artificial Sequence
  xmpE 2copy R (speI)
atgatactagtccttggggacttcgcgtgtcg

SEQ ID NO: 7 - DNA, 32 bp, Artificial Sequence
  xmpE 2copy F (speI)
atgatactagtctagatcttctcgacgggcag

SEQ ID NO: 8 - DNA, 20 bp, Artificial Sequence
  xmpE 2copy CF
ttcggctcagcattttccac

SEQ ID NO: 9 - DNA, 20 bp, Artificial Sequence
  xmpE 2copy CR
caatagtggtcgcgatgacg

SEQ ID NO: 10 - DNA, 36 bp, Artificial Sequence
  Pcj7 F
gcagtaaggagaatcagaaacatcccagcgctacta

SEQ ID NO: 11 - DNA, 40 bp, Artificial Sequence
  Pcj7 R
acctcttcggttgtgtgcacgagtgtttcctttcgttggg

SEQ ID NO: 12 - DNA, 31 bp, Artificial Sequence
  xmpE P 1
atgctctagatccagtgtggttaagaagtcg

SEQ ID NO: 13 - DNA, 33 bp, Artificial Sequence
  xmpE P 2
cgctgggatgtttctgattctccttactgcagt

SEQ ID NO: 14 - DNA, 43 bp, Artificial Sequence
  xmpE P 3
gtacccaacgaaaggaaacactcgtgcacacaaccgaagaggt

SEQ ID NO: 15 - DNA, 30 bp, Artificial Sequence
  xmpE P 4
atgctctagattattgagccagaaccatgg

SEQ ID NO: 16 - DNA, 21 bp, Artificial Sequence
  Pcj7/xmpE CF
ctagatcttctcgacgggcag

SEQ ID NO: 17 - DNA, 20 bp, Artificial Sequence
  Pcj7/xmpE CR
caatagtggtcgcgatgacg

SEQ ID NO: 18 - DNA, 31 bp, Artificial Sequence; identical to SEQ ID NO: 12
  xmpE atg 1

SEQ ID NO: 19 - DNA, 41 bp, Artificial Sequence
  xmpE atg 2
gacctcttcggttgtgtgcatgattctccttactgcagtta

SEQ ID NO: 20 - DNA, 41 bp, Artificial Sequence
  xmpE atg 3
taactgcagtaaggagaatcatgcacacaaccgaagaggtc

SEQ ID NO: 21 - DNA, 30 bp, Artificial Sequence
  xmpE atg 4
atgctctagactcgctcttgtcgacaacac